European Patent Application EP 4 253 560 A1, published October 4, 2023. Title: Enhanced detection of single-stranded nucleic acids using FokI-assisted digestion. Applicant: Consejo Superior de Investigaciones Científicas (CSIC). The sequence listing filed with the application follows.

SEQUENCE LISTING (79 sequences)

SEQ ID NO: 1 - DNA, 45 bp, Artificial Sequence
  Influenza A MB
tcttcggagacaatgcagacgaagagtcatccgacgtcggatgac

SEQ ID NO: 2 - DNA, 45 bp, Artificial Sequence
  Influenza B MB
tgtgactgtttcagtacgtgtcacagtcatccgacgtcggatgac

SEQ ID NO: 3 - DNA, 45 bp, Artificial Sequence
  Influenza C MB
agtgctttctcccttattgagcactgtcatccgacgtcggatgac

SEQ ID NO: 4 - DNA, 46 bp, Artificial Sequence
  Alphacoronavirus MB
gagactaaatgattactaaaagtctcgtcatccgacgtcggatgac

SEQ ID NO: 5 - DNA, 45 bp, Artificial Sequence
  Betacoronavirus (OC43/HKU1) MB
agcagaccttcctgagccttctgctgtcatccgacgtcggatgac

SEQ ID NO: 6 - DNA, 45 bp, Artificial Sequence
  SARS-CoV-2 (Spike) MB
tgctgattctcttcctgtttcagcagtcatccgacgtcggatgac

SEQ ID NO: 7 - DNA, 45 bp, Artificial Sequence
  SARS-CoV-2 (Orf8) MB
tgctgattttctagctccttcagcagtcatccgacgtcggatgac

SEQ ID NO: 8 - DNA, 45 bp, Artificial Sequence
  Rhinovirus MB
acccaaagtagttggtcccttgggtgtcatccgacgtcggatgac

SEQ ID NO: 9 - DNA, 45 bp, Artificial Sequence
  Parechovirus MB
gttacctacgggtaccttcggtaacgtcatccgacgtcggatgac

SEQ ID NO: 10 - DNA, 45 bp, Artificial Sequence
  Parainfluenza (Respirovirus/Rubulavirus) MB
tggttcaaggagacaatcagaaccagtcatccgacgtcggatgac

SEQ ID NO: 11 - DNA, 45 bp, Artificial Sequence
  Pneumovirus (Metapneumovirus/Orthopneumovirus) MB
ggtagaatgtttgctatgctctaccgtcatccgacgtcggatgac

SEQ ID NO: 12 - DNA, 30 bp, Artificial Sequence
  Influenza A DNA
tcgtactcctctgcattgtctccgaagaaa

SEQ ID NO: 13 - DNA, 30 bp, Artificial Sequence
  Influenza B DNA
atcccaaacgtactgaaacagtcacagcca

SEQ ID NO: 14 - DNA, 30 bp, Artificial Sequence
  Influenza C DNA
gaatctcaataagggagaaagcactgttga

SEQ ID NO: 15 - DNA, 32 bp, Artificial Sequence
  Alphacoronavirus DNA
ttgagttttagtaatcatttagtctcaactaa

SEQ ID NO: 16 - DNA, 30 bp, Artificial Sequence
  Betacoronavirus DNA
gttgaaggctcaggaaggtctgcttctaat

SEQ ID NO: 17 - DNA, 30 bp, Artificial Sequence
  SARS-CoV-2 (Spike) DNA
cttggaacaggaagagaatcagcaactgtg

SEQ ID NO: 18 - DNA, 30 bp, Artificial Sequence
  SARS-CoV-2 (Orf8)
agagtaggagctagaaaatcagcaccttta

SEQ ID NO: 19 - DNA, 30 bp, Artificial Sequence
  Rhinovirus DNA
cgggatgggaccaactactttgggtgtccg

SEQ ID NO: 20 - DNA, 30 bp, Artificial Sequence
  Parechovirus DNA
tgcccagaaggtacccgtaggtaacaagtg

SEQ ID NO: 21 - DNA, 29 bp, Artificial Sequence
  Parainfluenza DNA
atagcttgattgtctccttgaaccattgc

SEQ ID NO: 22 - DNA, 30 bp, Artificial Sequence
  Pneumovirus DNA
ttcctggttgcatagcaaacattctaccta

SEQ ID NO: 23 - RNA, 30 nt, Artificial Sequence
  Influenza A RNA
ucguacuccucugcauugucuccgaagaaa

SEQ ID NO: 24 - RNA, 30 nt, Artificial Sequence
  Influenza B RNA
aucccaaacguacugaaacagucacagcca

SEQ ID NO: 25 - RNA, 30 nt, Artificial Sequence
  Influenza C RNA
gaaucucaauaagggagaaagcacuguuga

SEQ ID NO: 26 - RNA, 32 nt, Artificial Sequence
  Alphacoronavirus RNA
uugaguuuuaguaaucauuuagucucaacuaa

SEQ ID NO: 27 - RNA, 30 nt, Artificial Sequence
  Betacoronavirus RNA
guugaaggcucaggaaggucugcuucuaau

SEQ ID NO: 28 - RNA, 30 nt, Artificial Sequence
  SARS-CoV-2 (Spike) RNA
cuuggaacaggaagagaaucagcaacugug

SEQ ID NO: 29 - RNA, 30 nt, Artificial Sequence
  SARS-CoV-2 (Orf8) RNA
agaguaggagcuagaaaaucagcaccuuua

SEQ ID NO: 30 - RNA, 30 nt, Artificial Sequence
  Rhinovirus RNA
cgggaugggaccaacuacuuuggguguccg

SEQ ID NO: 31 - RNA, 30 nt, Artificial Sequence
  Parechovirus RNA
ugcccagaagguacccguagguaacaagug

SEQ ID NO: 32 - RNA, 29 nt, Artificial Sequence
  Parainfluenza RNA
auagcuugauugucuccuugaaccauugc

SEQ ID NO: 33 - RNA, 30 nt, Artificial Sequence
  Pneumovirus RNA
uuccugguugcauagcaaacauucuaccua

SEQ ID NO: 34 - DNA, 78 bp, Artificial Sequence
  Influenza A Padlock probe
gcagaggagtacgacattatccctatagtgagtcgtattagaattttcccagtcgtacgcaattacttcggagacaat

SEQ ID NO: 35 - DNA, 78 bp, Artificial Sequence
  Influenza B Padlock probe
tcagtacgtttgggatattatccctatagtgagtcgtattagaattttccctggcatgaagaattggctgtgactgtt

SEQ ID NO: 36 - DNA, 78 bp, Artificial Sequence
  Influenza C Padlock probe
cttattgagattcacaattatccctatagtgagtcgtattagaattttcccagtcgttcaaacaacagtgctttctcc

SEQ ID NO: 37 - DNA, 78 bp, Artificial Sequence
  Alphacoronavirus Padlock probe
tactaaaactcaaacaattatccctatagtgagtcgtattagaattttcccttaggtacgcagttgagactaaatgat

SEQ ID NO: 38 - DNA, 78 bp, Artificial Sequence
  Betacoronavirus Padlock probe
cctgagccttcaacatattatccctatagtgagtcgtattagaattttcccagtcgtacgcaattagaagcagacctt

SEQ ID NO: 39 - DNA, 78 bp, Artificial Sequence
  SARS-CoV-2 (Spike) Padlock probe
gttccaagcataaacaattatccctatagtgagtcgtattagaattttcccagtcgtacgcatgctgattctcttcct

SEQ ID NO: 40 - DNA, 78 bp, Artificial Sequence
  SARS-CoV-2 (Orf8) Padlock probe
cctactctaatataccattatccctatagtgagtcgtattagaattttcccagtcgtacgcatgctgattttctagct

SEQ ID NO: 41 - DNA, 78 bp, Artificial Sequence
  Rhinovirus Padlock probe
gtcccgtcccatcccgattatccctatagtgagtcgtattagaattttcccagtcgtacggaacacccaaagtagttg

SEQ ID NO: 42 - DNA, 78 bp, Artificial Sequence
  Parechovirus Padlock probe
taccttctgggcatccattatccctatagtgagtcgtattagaatttagcatatccataccaacttgttacctacggg

SEQ ID NO: 43 - DNA, 78 bp, Artificial Sequence
  Parainfluenza Padlock probe
gacaatcaagctatagattatccctatagtgagtcgtattagaattttcccagtcgtacggatgcaatggttcaagga

SEQ ID NO: 44 - DNA, 78 bp, Artificial Sequence
  Pneumovirus Padlock probe
gctatgcaaccaggaaattatccctatagtgagtcgtattagaattatgccagtcgtacggatgtaggtagaatgttt

SEQ ID NO: 45 - DNA, 25 bp, Artificial Sequence
  Universal RCA primer
  modified_base (24)..(25): 3' - Phosphonothioate modification
aattctaatacgactcactataggg

SEQ ID NO: 46 - DNA, 45 bp, Artificial Sequence
  SARS-CoV-2 (strain B.1.1.7.) MB
gtaaccaagaccataagtgggttacgtcatccgacgtcggatgac

SEQ ID NO: 47 - DNA, 45 bp, Artificial Sequence
  SARS-CoV-2 (WT strain) MB
gtaaccaagaccattagtgggttacgtcatccgacgtcggatgac

SEQ ID NO: 48 - DNA, 30 bp, Artificial Sequence
  DNA 1 Watson (O1)
cagtcggatgacatgggtaccatcgtcatc

SEQ ID NO: 49 - DNA, 40 bp, Artificial Sequence
  DNA 1 Crick (O2)
ctagagatgacgatggtacccatgtcatccgactgcctac

SEQ ID NO: 50 - RNA, 40 nt, Artificial Sequence
  RNA 1 Crick (O3)
cuagagaugacgaugguacccaugucauccgacugccuac

SEQ ID NO: 51 - DNA, 30 bp, Artificial Sequence
  DNA 2 Watson (O4)
gtcagcctactgtacccatggtagcagtag

SEQ ID NO: 52 - DNA, 40 bp, Artificial Sequence
  DNA 2 Crick (O5)
gatctctactgctaccatgggtacagtaggctgacggatg

SEQ ID NO: 53 - RNA, 40 nt, Artificial Sequence
  RNA 2 Crick (O6)
gaucucuacugcuaccauggguacaguaggcugacggaug

SEQ ID NO: 54 - DNA, 36 bp, Artificial Sequence
  DNA 3 Watson (O7)
tgggtaccatcgtcatgtcatccgacgtcggatgac

SEQ ID NO: 55 - DNA, 46 bp, Artificial Sequence
  Fuel MB1 (O11)
tgctgagcagcctccatccactctgcgcagagtggatggaggctgc

SEQ ID NO: 56 - DNA, 43 bp, Artificial Sequence
  MB2 SARS-CoV-2 (Nsp4; O12)
tgctgatatgtccaaagtcagcagtcatccgacgtcggatgac

SEQ ID NO: 57 - DNA, 30 bp, Artificial Sequence
  DNA2 SARS-CoV-2 (Nsp4; O13)
attggtgctttggacatatcagcatctata

SEQ ID NO: 58 - RNA, 30 nt, Artificial Sequence
  RNA2 SARS-CoV-2 (Nsp4: O14)
auuggugcuuuggacauaucagcaucuaua

SEQ ID NO: 59 - DNA, 46 bp, Artificial Sequence
  MB1 MERS (Orf5; O18)
agtgagaacgcatgtcaaacctcactgtcatccgacgtcggatgac

SEQ ID NO: 60 - DNA, 30 bp, Artificial Sequence
  Control1 DNA SARS-CoV (O19)
catgggagagaaaaaaaatttctaattgtg

SEQ ID NO: 61 - DNA, 30 bp, Artificial Sequence
  Control1 DNA MERS (O20)
atttcaagcgtttggtttttaccaattgca

SEQ ID NO: 62 - DNA, 30 bp, Artificial Sequence
  Control DNA (O21)
tgctagaaaaccgcgtttctacgactggtg

SEQ ID NO: 63 - DNA, 30 bp, Artificial Sequence
  Control1 DNA SARS-CoV-2 (O22)
acttcagactattaccagctgtactcaact

SEQ ID NO: 64 - DNA, 30 bp, Artificial Sequence
  Control2 DNA SARS-Co-V (O23)
accgaagtttactaccagcttgagtctaca

SEQ ID NO: 65 - DNA, 30 bp, Artificial Sequence
  DNA4 MERS (Orf5; O24)
ccactgtttgacatgcgttctcactttatt

SEQ ID NO: 66 - RNA, 30 nt, Artificial Sequence
  Control1 RNA SARS-CoV (O25)
caugggagagaaaaaaaauuucuaauugug

SEQ ID NO: 67 - RNA, 30 nt, Artificial Sequence
  Control1 RNA MERS (O26)
auuucaagcguuugguuuuuaccaauugca

SEQ ID NO: 68 - RNA, 30 nt, Artificial Sequence
  Control RNA (O27)
ugcuagaaaaccgcguuucuacgacuggug

SEQ ID NO: 69 - RNA, 30 nt, Artificial Sequence
  Control2 RNA SARS-CoV-2 (O28)
acuucagacuauuaccagcuguacucaacu

SEQ ID NO: 70 - RNA, 30 nt, Artificial Sequence
  Control2 RNA SARS-CoV (O29)
accgaaguuuacuaccagcuugagucuaca

SEQ ID NO: 71 - RNA, 30 nt, Artificial Sequence
  RNA4 MERS (Orf5; O30)
ccacuguuugacaugcguucucacuuuauu

SEQ ID NO: 72 - DNA, 25 bp, Artificial Sequence
  RNA SC2 Wt (O33)
ccaacccactaatggtgttggttac

SEQ ID NO: 73 - DNA, 25 bp, Artificial Sequence
  RNA SC2 Mut (O34)
ccaacccacttatggtgttggttac

SEQ ID NO: 74 - DNA, 45 bp, Artificial Sequence
  MB1 SARSCOV2 (Spike) 11% 2OMe (O35)
  modified_base (8): um
  modified_base (9): cm
  modified_base (23): gm
  modified_base (24): cm
  modified_base (35): cm
tgctgatuctcttcctgtttcagcagtcatccgacgtcggatgac

SEQ ID NO: 75 - DNA, 45 bp, Artificial Sequence
  MB1 SARSCOV2 (Spike) 22% 2OMe (O36)
  modified_base (3): cm
  modified_base (7): um
  modified_base (9): cm
  modified_base (12): um
  modified_base (19): um
  modified_base (23): gm
  modified_base (26): gm
  modified_base (34): 2'-O-Methyladenosine
  modified_base (37): um
tgctgautctcutcctgtutcagcagtcatccgacgucggatgac

SEQ ID NO: 76 - DNA, 45 bp, Artificial Sequence
  MB1 SARSCOV2 (Spike) 62% 2OMe (O37)
  modified_base (1): um
  modified_base (2): gm
  modified_base (3): cm
  modified_base (4): um
  modified_base (5): gm
  modified_base (6): 2'-O-Methyladenosine
  modified_base (7): um
  modified_base (8): um
  modified_base (9): cm
  modified_base (10): um
  modified_base (11): cm
  modified_base (12): um
  modified_base (20): um
  modified_base (21): cm
  modified_base (22): 2'-O-Methyladenosine
  modified_base (23): gm
  modified_base (24): cm
  modified_base (25): 2 -O-methyladenosine
  modified_base (26): gm
  modified_base (27): um
  modified_base (33): gm
  modified_base (34): 2 -O-methyladenosine
  modified_base (35): cm
  modified_base (36): gm
  modified_base (37): um
  modified_base (38): cm
  modified_base (44): 2 -O-methyladenosine
  modified_base (45): cm
ugcugauucucutcctgttucagcagucatccgacgucggatgac

SEQ ID NO: 77 - DNA, 19 bp, Artificial Sequence
  2019-nCoV_N1-F (O41)
gaccccaaaatcagcgaat

SEQ ID NO: 78 - DNA, 24 bp, Artificial Sequence
  2019-nCoV_N1-R (O42)
tctggttactgccagttgaatctg

SEQ ID NO: 79 - DNA, 24 bp, Artificial Sequence
  2019-nCoV_N1-P-VIC (O43)
accccgcattacgtttggtggacc